European Patent Application EP 4 772 524 A1, published July 8, 2026. Title: Novel Peptide Having Activity of Improving Skin Condition and Uses Thereof. Applicant: CAREGEN CO., LTD. Application KR. The sequence listing filed with the application follows.

SEQUENCE LISTING (13 sequences)

SEQ ID NO: 1 - protein, 10 aa, synthetic construct
GRELVRAQIA

SEQ ID NO: 2 - DNA, 20 bp, synthetic construct
  source 1..20: mol_type = other DNA
caccctcaagagcctgagtc

SEQ ID NO: 3 - DNA, 20 bp, synthetic construct
  source 1..20: mol_type = other DNA
agacggctgagtagggaaca

SEQ ID NO: 4 - DNA, 20 bp, synthetic construct
  source 1..20: mol_type = other DNA
ccaggaaccgagtacaccat

SEQ ID NO: 5 - DNA, 20 bp, synthetic construct
  source 1..20: mol_type = other DNA
atacccaggttgggtgatga

SEQ ID NO: 6 - DNA, 20 bp, synthetic construct
  source 1..20: mol_type = other DNA
gcaagacctggctttggact

SEQ ID NO: 7 - DNA, 21 bp, synthetic construct
  source 1..21: mol_type = other DNA
gggagtttctggttagggctg

SEQ ID NO: 8 - DNA, 20 bp, synthetic construct
  source 1..20: mol_type = other DNA
ccttcttgggtgctggaata

SEQ ID NO: 9 - DNA, 20 bp, synthetic construct
  source 1..20: mol_type = other DNA
acacgataagggaggctgtg

SEQ ID NO: 10 - DNA, 20 bp, synthetic construct
  source 1..20: mol_type = other DNA
tcagtggctggaacagtgag

SEQ ID NO: 11 - DNA, 20 bp, synthetic construct
  source 1..20: mol_type = other DNA
tctggcatgtcccactatca

SEQ ID NO: 12 - DNA, 20 bp, synthetic construct
  source 1..20: mol_type = other DNA
ggagccaaaagggtcatcat

SEQ ID NO: 13 - DNA, 20 bp, synthetic construct
  source 1..20: mol_type = other DNA
gtgatggcatggactgtggt